European Patent Application EP 4 190 353 A1, published June 7, 2023. Title: ANTI-PD-1 ANTIBODY PHARMACEUTICAL COMPOSITION AND USE THEREOF. Applicant: Jiangsu Hengrui Pharmaceuticals Co., Ltd. Shanghai Hengrui Pharmaceutical Co., Ltd. Application EP 21849923.4. The sequence listing filed with the application follows.

SEQUENCE LISTING (82 sequences)

SEQ ID NO: 1 - protein, 401 aa, Artificial Sequence
  DOMAIN: Sequence of Human PD-1-IgG1Fc
MEFGLSWLFLVAILKGVQCPGWFLDSPDRPWNPPTFSPALLVVTEGDNATFTCSFSNTSESFVLNWYRMSPSNQTDKLAAFPEDRSQPGQDCRFRVTQLPNGRDFHMSVVRARRNDSGTYLCGAISLAPKAQIKESLRAELRVTERRAEVPTAHPSPSPRPAGQFQTLVEPKSSDKTHTCPPCPAPELLGGPSVFLFPPKPKDTLMISRTPEVTCVVVDVSHEDPEVKFNWYVDGVEVHNAKTKPREEQYNSTYRVVSVLTVLHQDWLNGKEYKCKVSNKALPAPIEKTISKAKGQPREPQVYTLPPSRDELTKNQVSLTCLVKGFYPSDIAVEWESNGQPENNYKTTPPVLDSDGSFFLYSKLTVDKSRWQQGNVFSCSVMHEALHNHYTQKSLSLSPGK

SEQ ID NO: 2 - protein, 186 aa, Artificial Sequence
  DOMAIN: Sequence of PD-1-his
MEFGLSWLFLVAILKGVQCPGWFLDSPDRPWNPPTFSPALLVVTEGDNATFTCSFSNTSESFVLNWYRMSPSNQTDKLAAFPEDRSQPGQDCRFRVTQLPNGRDFHMSVVRARRNDSGTYLCGAISLAPKAQIKESLRAELRVTERRAEVPTAHPSPSPRPAGQFQTLVGSSDYKDDDDKHHHHHH

SEQ ID NO: 3 - protein, 288 aa, Artificial Sequence
  DOMAIN: Sequence of PD-1 antigen transfecting cells
MQIPQAPWPVVWAVLQLGWRPGWFLDSPDRPWNPPTFSPALLVVTEGDNATFTCSFSNTSESFVLNWYRMSPSNQTDKLAAFPEDRSQPGQDCRFRVTQLPNGRDFHMSVVRARRNDSGTYLCGAISLAPKAQIKESLRAELRVTERRAEVPTAHPSPSPRPAGQFQTLVVGVVGGLLGSLVLLVWVLAVICSRAARGTIGARRTGQPLKEDPSAVPVFSVDYGELDFQWREKTPEPPVPCVPEQTEYATIVFPSGMGTSSPARRGSADGPRSAQPLRPEDGHCSWPL

SEQ ID NO: 4 - protein, 125 aa, Murine sequence (Mus musculus)
  DOMAIN: Heavy chain variable region sequence of M23
QVQLQQSGAELVRPGASVTLSCKASGYTFTDYEMHWVKQTPIHGLEWIGLIDPETGGTVYNQKFKDKTILTADKSSSTAYMEFRSLTSEDSAVYHCTRERFSYYGSTSDWYFDVWGTGTTVTVSS

SEQ ID NO: 5 - protein, 112 aa, Murine sequence (Mus musculus)
  DOMAIN: Light chain variable region sequence of M23
DGLMTQTPLSLPVSLGDHASISCRSSQSLVHSNGNTYLEWYLQKPGQSPKLLIYKVSNRFSGVPDRFSGSGSGTDFTLKISRVEAEDLGIYYCFQGSHVPYTFGGGTKLEIK

SEQ ID NO: 6 - protein, 120 aa, Murine sequence (Mus musculus)
  DOMAIN: Heavy chain variable region sequence of M32
QVQLQQSGAELVRPGASVTLSCKASDFTFTDYEIHWVKQTPVHGLEWIGLFDPETGGIVYNQKFKGKAILTADKSSNTAYMEFRSLTSEDSAVYYCTREGYNRDWYFDVWGTGTTVTVSS

SEQ ID NO: 7 - protein, 112 aa, Murine sequence (Mus musculus)
  DOMAIN: Light chain variable region sequence of M32
DVLMTQTPLSLPVSLGDQASISCRSSQSIVHSNGNTYLEWYLQKPGQSPKLLIYKVSNRFSGVPDRFSGSGSGTDFTLKISRVEAEDLGIYYCFQGSHVPYAFGGGTKLEIK

SEQ ID NO: 8 - protein, 5 aa, Murine sequence (Mus musculus)
  DOMAIN: HCDR1 sequence of M23
DYEMH

SEQ ID NO: 9 - protein, 17 aa, Murine sequence (Mus musculus)
  DOMAIN: HCDR2 sequence of M23
LIDPETGGTVYNQKFKD

SEQ ID NO: 10 - protein, 16 aa, Murine sequence (Mus musculus)
  DOMAIN: HCDR3 sequence of M23
ERFSYYGSTSDWYFDV

SEQ ID NO: 11 - protein, 16 aa, Murine sequence (Mus musculus)
  DOMAIN: LCDR1 sequence of M23
RSSQSLVHSNGKTYLE

SEQ ID NO: 12 - protein, 7 aa, Murine sequence (Mus musculus)
  DOMAIN: LCDR2 sequence of M23/M32
KVSNRFS

SEQ ID NO: 13 - protein, 9 aa, Murine sequence (Mus musculus)
  DOMAIN: LCDR3 sequence of M23
FQGSHVPYT

SEQ ID NO: 14 - protein, 5 aa, Murine sequence (Mus musculus)
  DOMAIN: HCDR1 sequence of M32
DYEIH

SEQ ID NO: 15 - protein, 17 aa, Murine sequence (Mus musculus)
  DOMAIN: HCDR2 sequence of M32
LFDPETGGIVYNQKFKG

SEQ ID NO: 16 - protein, 11 aa, Murine sequence (Mus musculus)
  DOMAIN: HCDR3 sequence of M32
EGYNRDWYFDV

SEQ ID NO: 17 - protein, 16 aa, Murine sequence (Mus musculus)
  DOMAIN: LCDR1 sequence of M32
RSSQSIVHSNGNTYLE

SEQ ID NO: 18 - protein, 9 aa, Murine sequence (Mus musculus)
  DOMAIN: LCDR3 sequence of M32
FQGSHVPYA

SEQ ID NO: 19 - protein, 118 aa, Murine sequence (Mus musculus)
  DOMAIN: Heavy chain variable region sequence of M33
KVMLVESGGGLVKPGGSLKLSCAASGFTFSSYAMSWVRQTPEKRLEWVATISGGGVDTYYQDNVQGRFTISRDNAKNTLYLQMSSLRSEDTALYYCASPYGHGYFDVWGTGTTVTVSS

SEQ ID NO: 20 - protein, 107 aa, Murine sequence (Mus musculus)
  DOMAIN: Light chain variable region sequence of M33
DIQMTQTTSSLSASLGDRVTISCRASQDINNFLNWYQQKPDGTVKLLIYYTSSLHSGVPSRFSGSGSGTDYSLTISNLEQEDIATYFCQQGNTLPWTFGGGTKLEIK

SEQ ID NO: 21 - protein, 5 aa, Murine sequence (Mus musculus)
  DOMAIN: HCDR1 sequence of M33
SYAMS

SEQ ID NO: 22 - protein, 17 aa, Murine sequence (Mus musculus)
  DOMAIN: HCDR2 sequence of M33
TISGGGVDTYYQDNVQG

SEQ ID NO: 23 - protein, 9 aa, Murine sequence (Mus musculus)
  DOMAIN: HCDR3 sequence of M33
PYGHGYFDV

SEQ ID NO: 24 - protein, 11 aa, Murine sequence (Mus musculus)
  DOMAIN: LCDR1 sequence of M33
RASQDINNFLN

SEQ ID NO: 25 - protein, 7 aa, Murine sequence (Mus musculus)
  DOMAIN: LCDR2 sequence of M33
YTSSLHS

SEQ ID NO: 26 - protein, 9 aa, Murine sequence (Mus musculus)
  DOMAIN: LCDR3 sequence of M33
QQGNTLPWT

SEQ ID NO: 27 - protein, 125 aa, Artificial Sequence
  DOMAIN: Sequence of Hu23VH1/Hu23VH-CDR grafted
EVQLVQSGAEVKKPGSSVKVSCKASGGTFSDYEMHWVRQAPGQGLEWMGLIDPETGGTVYNQKFKDRVTITADKSTSTAYMELSSLRSEDTAVYYCARERFSYYGSTSDWYFDVWGQGTTVTVSS

SEQ ID NO: 28 - protein, 112 aa, Artificial Sequence
  DOMAIN: Sequence of Hu23VL1/Hu23VL-CDR grafted
DIVMTQTPLSLPVTPGEPASISCRSSQSLVHSNGNTYLEWYLQKPGQSPQLLIYKVSNRFSGVPDRFSGSGSGTDFTLKISRVEAEDVGVYYCFQGSHVPYTFGGGTKVEIK

SEQ ID NO: 29 - protein, 112 aa, Artificial Sequence
  DOMAIN: Sequence of Hu23VL2
DGVMTQTPLSLPVTPGEPASISCRSSQSLVHSNGNTYLEWYLQKPGQSPQLLIYKVSNRFSGVPDRFSGSGSGTDFTLKISRVEAEDVGVYYCFQGSHVPYTFGGGTKVEIK

SEQ ID NO: 30 - protein, 125 aa, Artificial Sequence
  DOMAIN: Sequence of Hu23VH2
EVQLVQSGAEVKKPGSSVKVSCKASGYTFSDYEMHWVRQAPGQGLEWMGLIDPETGGTVYNQKFKDRVTLTADKSTSTAYMELSSLRSEDTAVYYCARERFSYYGSTSDWYFDVWGQGTTVTVSS

SEQ ID NO: 31 - protein, 125 aa, Artificial Sequence
  DOMAIN: Sequence of Hu23VH3
EVQLVQSGAEVKKPGSSVKVSCKASGYTFSDYEMHWVRQAPGQGLEWIGLIDPETGGTVYNQKFKDRTTLTADKSTSTAYMEFSSLRSEDTAVYYCARERFSYYGSTSDWYFDVWGQGTTVTVSS

SEQ ID NO: 32 - protein, 125 aa, Artificial Sequence
  DOMAIN: Sequence of Hu23VH4
EVQLVQSGAEVKKPGSSVKVSCKASGYTFSDYEMHWVRQAPGQGLEWIGLIDPETGGTVYNQKFKDRTTLTADKSTSTAYMEFSSLRSEDTAVYYCTRERFSYYGSTSDWYFDVWGQGTTVTVSS

SEQ ID NO: 33 - protein, 120 aa, Artificial Sequence
  DOMAIN: Sequence of Hu32VH1/Hu32VH-CDR grafted
EVQLVQSGAEVKKPGSSVKVSCKASGGTFSDYEIHWVRQAPGQGLEWMGLFDPETGGIVYNQKFKGRVTITADKSTSTAYMELSSLRSEDTAVYYCAREGYNRDWYFDVWGQGTTVTVSS

SEQ ID NO: 34 - protein, 112 aa, Artificial Sequence
  DOMAIN: Sequence of Hu32VL1/Hu32VL-CDR grafted
DIVMTQTPLSLPVTPGEPASISCRSSQSIVHSNGNTYLEWYLQKPGQSPQLLIYKVSNRFSGVPDRFSGSGSGTDFTLKISRVEAEDVGVYYCFQGSHVPYAFGGGTKVEIK

SEQ ID NO: 35 - protein, 112 aa, Artificial Sequence
  DOMAIN: Sequence of Hu32VL2
DVVMTQTPLSLPVTPGEPASISCRSSQSIVHSNGNTYLEWYLQKPGQSPQLLIYKVSNRFSGVPDRFSGSGSGTDFTLKISRVEAEDVGVYYCFQGSHVPYAFGGGTKVEIK

SEQ ID NO: 36 - protein, 120 aa, Artificial Sequence
  DOMAIN: Sequence of Hu32VH2
EVQLVQSGAEVKKPGSSVKVSCKASGFTFSDYEIHWVRQAPGQGLEWMGLFDPETGGIVYNQKFKGRVTLTADKSTSTAYMELSSLRSEDTAVYYCTREGYNRDWYFDVWGQGTTVTVSS

SEQ ID NO: 37 - protein, 120 aa, Artificial Sequence
  DOMAIN: Sequence of Hu32VH3
EVQLVQSGAEVKKPGSSVKVSCKASDFTFSDYEIHWVRQAPGQGLEWMGLFDPETGGIVYNQKFKGRVTLTADKSTSTAYMELSSLRSEDTAVYYCTREGYNRDWYFDVWGQGTTVTVSS

SEQ ID NO: 38 - protein, 120 aa, Artificial Sequence
  DOMAIN: Sequence of Hu32VH4
EVQLVQSGAEVKKPGSSVKVSCKASGFTFSDYEIHWVRQAPGQGLEWIGLFDPETGGIVYNQKFKGRATLTADKSTSTAYMEFSSLRSEDTAVYYCTREGYNRDWYFDVWGQGTTVTVSS

SEQ ID NO: 39 - protein, 120 aa, Artificial Sequence
  DOMAIN: Sequence of Hu32VH5
EVQLVQSGAEVKKPGSSVKVSCKASDFTFTDYEIHWVRQAPGQGLEWIGLFDPETGGIVYNQKFKGRATLTADKSTSTAYMEFSSLRSEDTAVYYCTREGYNRDWYFDVWGQGTTVTVSS

SEQ ID NO: 40 - protein, 120 aa, Artificial Sequence
  DOMAIN: Sequence of Hu32VH6
EVQLVQSGAEVKKPGSSVKVSCKASDFTFTDYEIHWVKQAPGHGLEWIGLFDPETGGIVYNQKFKGKATLTADKSTSTAYMEFSSLRSEDTAVYYCTREGYNRDWYFDVWGQGTTVTVSS

SEQ ID NO: 41 - protein, 118 aa, Artificial Sequence
  DOMAIN: Sequence of Hu33VH1/Hu33VH-CDR grafted
EVQLVESGGGLVQPGGSLRLSCAASGFTFSSYAMSWVRQAPGKGLEWVATISGGGVDTYYQDNVQGRFTISRDNAKNSLYLQMNSLRAEDTAVYYCARPYGHGYFDVWGQGTTVTVSS

SEQ ID NO: 42 - protein, 107 aa, Artificial Sequence
  DOMAIN: Sequence of Hu33VL1/Hu33VL-CDR grafted
DIQMTQSPSSLSASVGDRVTITCRASQDINNFLNWYQQKPGKAPKLLIYYTSSLHSGVPSRFSGSGSGTDFTLTISSLQPEDFATYYCQQGNTLPWTFGGGTKVEIK

SEQ ID NO: 43 - protein, 107 aa, Artificial Sequence
  DOMAIN: Sequence of Hu33VL2
DIQMTQSPSSLSASVGDRVTITCRASQDINNFLNWYQQKPGKAPKLLIYYTSSLHSGVPSRFSGSGSGTDYTLTISSLQPEDFATYYCQQGNTLPWTFGGGTKVEIK

SEQ ID NO: 44 - protein, 107 aa, Artificial Sequence
  DOMAIN: Sequence of Hu33VL3
DIQMTQSPSSLSASVGDRVTITCRASQDINNFLNWYQQKPGGAVKLLIYYTSSLHSGVPSRFSGSGSGTDYTLTISSLQPEDFATYYCQQGNTLPWTFGGGTKVEIK

SEQ ID NO: 45 - protein, 118 aa, Artificial Sequence
  DOMAIN: Sequence of Hu33VH2
EVQLVESGGGLVQPGGSLRLSCAASGFTFSSYAMSWVRQAPGKGLEWVATISGGGVDTYYQDNVQGRFTISRDNAKNSLYLQMNSLRAEDTAVYYCASPYGHGYFDVWGQGTTVTVSS

SEQ ID NO: 46 - protein, 118 aa, Artificial Sequence
  DOMAIN: Sequence of Hu33VH3
KVQLVESGGGLVQPGGSLRLSCAASGFTFSSYAMSWVRQAPGKGLEWVATISGGGVDTYYQDNVQGRFTISRDNAKNSLYLQMNSLRAEDTAVYYCASPYGHGYFDVWGQGTTVTVSS

SEQ ID NO: 47 - protein, 16 aa, Artificial Sequence
  DOMAIN: Sequence of Hu23LCDR1(N28Q)
RSSQSLVHSQGNTYLE

SEQ ID NO: 48 - protein, 16 aa, Artificial Sequence
  DOMAIN: Sequence of Hu23LCDR1(N28L)
RSSQSLVHSLGNTYLE

SEQ ID NO: 49 - protein, 16 aa, Artificial Sequence
  DOMAIN: Sequence of Hu23LCDR1(N28T)
RSSQSLVHSTGNTYLE

SEQ ID NO: 50 - protein, 16 aa, Artificial Sequence
  DOMAIN: Sequence of Hu23LCDR1(N28D)
RSSQSLVHSDGNTYLE

SEQ ID NO: 51 - protein, 16 aa, Artificial Sequence
  DOMAIN: Sequence of Hu23LCDR1(G29A)
RSSQSLVHSNANTYLE

SEQ ID NO: 52 - protein, 16 aa, Artificial Sequence
  DOMAIN: Sequence of Hu23LCDR1(G29V)
RSSQSLVHSNVNTYLE

SEQ ID NO: 53 - protein, 112 aa, Artificial Sequence
  DOMAIN: Sequence of Hu23VL1(N28Q)
DIVMTQTPLSLPVTPGEPASISCRSSQSLVHSQGNTYLEWYLQKPGQSPQLLIYKVSNRFSGVPDRFSGSGSGTDFTLKISRVEAEDVGVYYCFQGSHVPYTFGGGTKVEIK

SEQ ID NO: 54 - protein, 112 aa, Artificial Sequence
  DOMAIN: Sequence of Hu23VL1(N28L)
DIVMTQTPLSLPVTPGEPASISCRSSQSLVHSLGNTYLEWYLQKPGQSPQLLIYKVSNRFSGVPDRFSGSGSGTDFTLKISRVEAEDVGVYYCFQGSHVPYTFGGGTKVEIK

SEQ ID NO: 55 - protein, 112 aa, Artificial Sequence
  DOMAIN: Sequence of Hu23VL1(N28T)
DIVMTQTPLSLPVTPGEPASISCRSSQSLVHSTGNTYLEWYLQKPGQSPQLLIYKVSNRFSGVPDRFSGSGSGTDFTLKISRVEAEDVGVYYCFQGSHVPYTFGGGTKVEIK

SEQ ID NO: 56 - protein, 112 aa, Artificial Sequence
  DOMAIN: Sequence of Hu23VL1(N28D)
DIVMTQTPLSLPVTPGEPASISCRSSQSLVHSDGNTYLEWYLQKPGQSPQLLIYKVSNRFSGVPDRFSGSGSGTDFTLKISRVEAEDVGVYYCFQGSHVPYTFGGGTKVEIK

SEQ ID NO: 57 - protein, 112 aa, Artificial Sequence
  DOMAIN: Sequence of Hu23VL1(G29A)
DIVMTQTPLSLPVTPGEPASISCRSSQSLVHSNANTYLEWYLQKPGQSPQLLIYKVSNRFSGVPDRFSGSGSGTDFTLKISRVEAEDVGVYYCFQGSHVPYTFGGGTKVEIK

SEQ ID NO: 58 - protein, 112 aa, Artificial Sequence
  DOMAIN: Sequence of Hu23VL1(G29V)
DIVMTQTPLSLPVTPGEPASISCRSSQSLVHSNVNTYLEWYLQKPGQSPQLLIYKVSNRFSGVPDRFSGSGSGTDFTLKISRVEAEDVGVYYCFQGSHVPYTFGGGTKVEIK

SEQ ID NO: 59 - protein, 112 aa, Artificial Sequence
  DOMAIN: Sequence of Hu23VL2(N28Q)
DGVMTQTPLSLPVTPGEPASISCRSSQSLVHSQGNTYLEWYLQKPGQSPQLLIYKVSNRFSGVPDRFSGSGSGTDFTLKISRVEAEDVGVYYCFQGSHVPYTFGGGTKVEIK

SEQ ID NO: 60 - protein, 112 aa, Artificial Sequence
  DOMAIN: Sequence of Hu23VL2(N28L)
DGVMTQTPLSLPVTPGEPASISCRSSQSLVHSLGNTYLEWYLQKPGQSPQLLIYKVSNRFSGVPDRFSGSGSGTDFTLKISRVEAEDVGVYYCFQGSHVPYTFGGGTKVEIK

SEQ ID NO: 61 - protein, 112 aa, Artificial Sequence
  DOMAIN: Sequence of Hu23VL2(N28T)
DGVMTQTPLSLPVTPGEPASISCRSSQSLVHSTGNTYLEWYLQKPGQSPQLLIYKVSNRFSGVPDRFSGSGSGTDFTLKISRVEAEDVGVYYCFQGSHVPYTFGGGTKVEIK

SEQ ID NO: 62 - protein, 112 aa, Artificial Sequence
  DOMAIN: Sequence of Hu23VL2(N28D)
DGVMTQTPLSLPVTPGEPASISCRSSQSLVHSDGNTYLEWYLQKPGQSPQLLIYKVSNRFSGVPDRFSGSGSGTDFTLKISRVEAEDVGVYYCFQGSHVPYTFGGGTKVEIK

SEQ ID NO: 63 - protein, 112 aa, Artificial Sequence
  DOMAIN: Sequence of Hu23VL2(G29A)
DGVMTQTPLSLPVTPGEPASISCRSSQSLVHSNANTYLEWYLQKPGQSPQLLIYKVSNRFSGVPDRFSGSGSGTDFTLKISRVEAEDVGVYYCFQGSHVPYTFGGGTKVEIK

SEQ ID NO: 64 - protein, 112 aa, Artificial Sequence
  DOMAIN: Sequence of Hu23VL2(G29V)
DGVMTQTPLSLPVTPGEPASISCRSSQSLVHSNVNTYLEWYLQKPGQSPQLLIYKVSNRFSGVPDRFSGSGSGTDFTLKISRVEAEDVGVYYCFQGSHVPYTFGGGTKVEIK

SEQ ID NO: 65 - protein, 5 aa, Artificial Sequence
  DOMAIN: Sequence of HCDR1 general formula of Hu32 and Hu23 antibodies
  DOMAIN (4)..(4): Xaa is selected from the group consisting of Ile and Met
DYEXH

SEQ ID NO: 66 - protein, 17 aa, Artificial Sequence
  DOMAIN: Sequence of HCDR2 general formula of Hu32 and Hu23 antibodies
  DOMAIN (2)..(2): Xaa is selected from the group consisting of Phe and Ile
  DOMAIN (9)..(9): Xaa is selected from the group consisting of Ile and Thr
  DOMAIN (17)..(17): Xaa is selected from the group consisting of Gly and Asp
LXDPETGGXVYNQKFKX

SEQ ID NO: 67 - protein, 16 aa, Artificial Sequence
  DOMAIN: Sequence of HCDR3 general formula of Hu32 and Hu23 antibodies
  DOMAIN (2)..(2): Xaa is selected from the group consisting of Gly and Arg
  DOMAIN (3)..(3): Xaa is Phe or vacancy
  DOMAIN (4)..(4): Xaa is Ser or vacancy
  DOMAIN (5)..(5): Xaa is Tyr or vacancy
  DOMAIN (7)..(7): Xaa is Gly or vacancy
  DOMAIN (8)..(8): Xaa is Ser or vacancy
  DOMAIN (9)..(9): Xaa is selected from the group consisting of Asn and Thr
  DOMAIN (10)..(10): Xaa is selected from the group consisting of Arg and Ser
EXXXXYXXXXDWYFDV

SEQ ID NO: 68 - protein, 16 aa, Artificial Sequence
  DOMAIN: Sequence of LCDR1 general formula of Hu32 and Hu23 antibodies
  DOMAIN (6)..(6): Xaa is selected from the group consisting of Ile and Leu
  DOMAIN (10)..(10): Xaa is selected from the group consisting of Asn, Gln, Leu, Thr and Asp
  DOMAIN (11)..(11): Xaa is selected from the group consisting of Gly, Ala and Val
  DOMAIN (12)..(12): Xaa is selected from the group consisting of Asn and Lys
RSSQSXVHSXXXTYLE

SEQ ID NO: 69 - protein, 9 aa, Artificial Sequence
  DOMAIN: Sequence of LCDR3 general formula of Hu32 and Hu23 antibodies
  DOMAIN (9)..(9): Xaa is selected from the group consisting of Ala and Thr
FQGSHVPYX

SEQ ID NO: 70 - protein, 125 aa, Artificial Sequence
  DOMAIN: Sequence of heavy chain variable region general formula of Hu32 and Hu23 antibodies
  DOMAIN (26)..(26): Xaa is selected from the group consisting of Gly and Asp
  DOMAIN (27)..(27): Xaa is selected from the group consisting of Gly, Phe and Tyr
  DOMAIN (30)..(30): Xaa is selected from the group consisting of Ser and Thr
  DOMAIN (34)..(34): Xaa is selected from the group consisting of Ile and Met
  DOMAIN (38)..(38): Xaa is selected from the group consisting of Arg and Lys
  DOMAIN (43)..(43): Xaa is selected from the group consisting of Gln and His
  DOMAIN (48)..(48): Xaa is selected from the group consisting of Ile and Met
  DOMAIN (51)..(51): Xaa is selected from the group consisting of Phe and Ile
  DOMAIN (58)..(58): Xaa is selected from the group consisting of Ile and Thr
  DOMAIN (66)..(66): Xaa is selected from the group consisting of Gly and Asp
  DOMAIN (67)..(67): Xaa is selected from the group consisting of Arg and Lys
  DOMAIN (68)..(68): Xaa is selected from the group consisting of Val, Ala and Thr
  DOMAIN (70)..(70): Xaa is selected from the group consisting of Arg and Lys
  DOMAIN (83)..(83): Xaa is selected from the group consisting of Leu and Phe
  DOMAIN (97)..(97): Xaa is selected from the group consisting of Ala and Thr
  DOMAIN (100)..(100): Xaa is selected from the group consisting of Gly and Arg
  DOMAIN (101)..(101): Xaa is Phe or vacancy
  DOMAIN (102)..(102): Xaa is Ser or vacancy
  DOMAIN (103)..(103): Xaa is Tyr or vacancy
  DOMAIN (105)..(105): Xaa is Gly or vacancy
  DOMAIN (106)..(106): Xaa is Ser or vacancy
  DOMAIN (107)..(107): Xaa is selected from the group consisting of Asn and Thr
  DOMAIN (108)..(108): Xaa is selected from the group consisting of Arg and Ser
EVQLVQSGAEVKKPGSSVKVSCKASXXTFXDYEXHWVXQAPGXGLEWXGLXDPETGGXVYNQKFKXXXTXTADKSTSTAYMEXSSLRSEDTAVYYCXREXXXXYXXXXDWYFDVWGQGTTVTVSS

SEQ ID NO: 71 - protein, 112 aa, Artificial Sequence
  DOMAIN: Sequence of light chain variable region general formula of Hu32 and Hu23 antibodies
  DOMAIN (2)..(2): Xaa is selected from the group consisting of Ile, Val and Gly
  DOMAIN (29)..(29): Xaa is selected from the group consisting of Ile and Leu
  DOMAIN (33)..(33): Xaa is selected from the group consisting of Asn, Gln, Leu, Thr and Asp
  DOMAIN (34)..(34): Xaa is selected from the group consisting of Gly, Ala and Val
  DOMAIN (35)..(35): Xaa is selected from the group consisting of Asn and Lys
  DOMAIN (102)..(102): Xaa is selected from the group consisting of Ala and Thr
DXVMTQTPLSLPVTPGEPASISCRSSQSXVHSXXXTYLEWYLQKPGQSPQLLIYKVSNRFSGVPDRFSGSGSGTDFTLKISRVEAEDVGVYYCFQGSHVPYXFGGGTKVEIK

SEQ ID NO: 72 - protein, 327 aa, Artificial Sequence
  DOMAIN: Heavy chain constant region sequence of IgG4-AA
ASTKGPSVFPLAPCSRSTSESTAALGCLVKDYFPEPVTVSWNSGALTSGVHTFPAVLQSSGLYSLSSVVTVPSSSLGTKTYTCNVDHKPSNTKVDKRVESKYGPPCPPCPAPEAAGGPSVFLFPPKPKDTLMISRTPEVTCVVVDVSQEDPEVQFNWYVDGVEVHNAKTKPREEQFNSTYRVVSVLTVLHQDWLNGKEYKCKVSNKGLPSSIEKTISKAKGQPREPQVYTLPPSQEEMTKNQVSLTCLVKGFYPSDIAVEWESNGQPENNYKTTPPVLDSDGSFFLYSRLTVDKSRWQEGNVFSCSVMHEALHNHYTQKSLSLSLGK

SEQ ID NO: 73 - protein, 107 aa, Artificial Sequence [sequence omitted]

SEQ ID NO: 74 - protein, 452 aa, Artificial Sequence
  CHAIN: Heavy chain sequence of Hu23-11.IgG4AA antibody
EVQLVQSGAEVKKPGSSVKVSCKASGGTFSDYEMHWVRQAPGQGLEWMGLIDPETGGTVYNQKFKDRVTITADKSTSTAYMELSSLRSEDTAVYYCARERFSYYGSTSDWYFDVWGQGTTVTVSSASTKGPSVFPLAPCSRSTSESTAALGCLVKDYFPEPVTVSWNSGALTSGVHTFPAVLQSSGLYSLSSVVTVPSSSLGTKTYTCNVDHKPSNTKVDKRVESKYGPPCPPCPAPEAAGGPSVFLFPPKPKDTLMISRTPEVTCVVVDVSQEDPEVQFNWYVDGVEVHNAKTKPREEQFNSTYRVVSVLTVLHQDWLNGKEYKCKVSNKGLPSSIEKTISKAKGQPREPQVYTLPPSQEEMTKNQVSLTCLVKGFYPSDIAVEWESNGQPENNYKTTPPVLDSDGSFFLYSRLTVDKSRWQEGNVFSCSVMHEALHNHYTQKSLSLSLGK

SEQ ID NO: 75 - protein, 219 aa, Artificial Sequence
  CHAIN: Light chain sequence of Hu23-11.IgG4AA/Hu32a-85.IgG4AA/Hu23-11.IgG4P/Hu32a-85.IgG4P
DIVMTQTPLSLPVTPGEPASISCRSSQSLVHSTGNTYLEWYLQKPGQSPQLLIYKVSNRFSGVPDRFSGSGSGTDFTLKISRVEAEDVGVYYCFQGSHVPYTFGGGTKVEIKRTVAAPSVFIFPPSDEQLKSGTASVVCLLNNFYPREAKVQWKVDNALQSGNSQESVTEQDSKDSTYSLSSTLTLSKADYEKHKVYACEVTHQGLSSPVTKSFNRGEC

SEQ ID NO: 76 - protein, 447 aa, Artificial Sequence
  CHAIN: Heavy chain sequence of Hu32a-85.IgG4AA
EVQLVQSGAEVKKPGSSVKVSCKASDFTFTDYEIHWVKQAPGHGLEWIGLFDPETGGIVYNQKFKGKATLTADKSTSTAYMEFSSLRSEDTAVYYCTREGYNRDWYFDVWGQGTTVTVSSASTKGPSVFPLAPCSRSTSESTAALGCLVKDYFPEPVTVSWNSGALTSGVHTFPAVLQSSGLYSLSSVVTVPSSSLGTKTYTCNVDHKPSNTKVDKRVESKYGPPCPPCPAPEAAGGPSVFLFPPKPKDTLMISRTPEVTCVVVDVSQEDPEVQFNWYVDGVEVHNAKTKPREEQFNSTYRVVSVLTVLHQDWLNGKEYKCKVSNKGLPSSIEKTISKAKGQPREPQVYTLPPSQEEMTKNQVSLTCLVKGFYPSDIAVEWESNGQPENNYKTTPPVLDSDGSFFLYSRLTVDKSRWQEGNVFSCSVMHEALHNHYTQKSLSLSLGK

SEQ ID NO: 77 - protein, 445 aa, Artificial Sequence
  CHAIN: Heavy chain sequence of Hu33-6.IgG4AA
KVQLVESGGGLVQPGGSLRLSCAASGFTFSSYAMSWVRQAPGKGLEWVATISGGGVDTYYQDNVQGRFTISRDNAKNSLYLQMNSLRAEDTAVYYCASPYGHGYFDVWGQGTTVTVSSASTKGPSVFPLAPCSRSTSESTAALGCLVKDYFPEPVTVSWNSGALTSGVHTFPAVLQSSGLYSLSSVVTVPSSSLGTKTYTCNVDHKPSNTKVDKRVESKYGPPCPPCPAPEAAGGPSVFLFPPKPKDTLMISRTPEVTCVVVDVSQEDPEVQFNWYVDGVEVHNAKTKPREEQFNSTYRVVSVLTVLHQDWLNGKEYKCKVSNKGLPSSIEKTISKAKGQPREPQVYTLPPSQEEMTKNQVSLTCLVKGFYPSDIAVEWESNGQPENNYKTTPPVLDSDGSFFLYSRLTVDKSRWQEGNVFSCSVMHEALHNHYTQKSLSLSLGK

SEQ ID NO: 78 - protein, 214 aa, Artificial Sequence
  CHAIN: Light chain sequence of Hu33-6.IgG4AA/Hu33-6.IgG4P
DIQMTQSPSSLSASVGDRVTITCRASQDINNFLNWYQQKPGKAPKLLIYYTSSLHSGVPSRFSGSGSGTDYTLTISSLQPEDFATYYCQQGNTLPWTFGGGTKVEIKRTVAAPSVFIFPPSDEQLKSGTASVVCLLNNFYPREAKVQWKVDNALQSGNSQESVTEQDSKDSTYSLSSTLTLSKADYEKHKVYACEVTHQGLSSPVTKSFNRGEC

SEQ ID NO: 79 - protein, 327 aa, Artificial Sequence
  DOMAIN: Heavy chain constant region sequence of IgG4-P
ASTKGPSVFPLAPCSRSTSESTAALGCLVKDYFPEPVTVSWNSGALTSGVHTFPAVLQSSGLYSLSSVVTVPSSSLGTKTYTCNVDHKPSNTKVDKRVESKYGPPCPPCPAPEFLGGPSVFLFPPKPKDTLMISRTPEVTCVVVDVSQEDPEVQFNWYVDGVEVHNAKTKPREEQFNSTYRVVSVLTVLHQDWLNGKEYKCKVSNKGLPSSIEKTISKAKGQPREPQVYTLPPSQEEMTKNQVSLTCLVKGFYPSDIAVEWESNGQPENNYKTTPPVLDSDGSFFLYSRLTVDKSRWQEGNVFSCSVMHEALHNHYTQKSLSLSLGK

SEQ ID NO: 80 - protein, 452 aa, Artificial Sequence
  CHAIN: Heavy chain sequence of Hu23-11. IgG4P antibody
EVQLVQSGAEVKKPGSSVKVSCKASGGTFSDYEMHWVRQAPGQGLEWMGLIDPETGGTVYNQKFKDRVTITADKSTSTAYMELSSLRSEDTAVYYCARERFSYYGSTSDWYFDVWGQGTTVTVSSASTKGPSVFPLAPCSRSTSESTAALGCLVKDYFPEPVTVSWNSGALTSGVHTFPAVLQSSGLYSLSSVVTVPSSSLGTKTYTCNVDHKPSNTKVDKRVESKYGPPCPPCPAPEFLGGPSVFLFPPKPKDTLMISRTPEVTCVVVDVSQEDPEVQFNWYVDGVEVHNAKTKPREEQFNSTYRVVSVLTVLHQDWLNGKEYKCKVSNKGLPSSIEKTISKAKGQPREPQVYTLPPSQEEMTKNQVSLTCLVKGFYPSDIAVEWESNGQPENNYKTTPPVLDSDGSFFLYSRLTVDKSRWQEGNVFSCSVMHEALHNHYTQKSLSLSLGK

SEQ ID NO: 81 - protein, 447 aa, Artificial Sequence
  CHAIN: Heavy chain sequence of Hu32a-85. IgG4P
EVQLVQSGAEVKKPGSSVKVSCKASDFTFTDYEIHWVKQAPGHGLEWIGLFDPETGGIVYNQKFKGKATLTADKSTSTAYMEFSSLRSEDTAVYYCTREGYNRDWYFDVWGQGTTVTVSSASTKGPSVFPLAPCSRSTSESTAALGCLVKDYFPEPVTVSWNSGALTSGVHTFPAVLQSSGLYSLSSVVTVPSSSLGTKTYTCNVDHKPSNTKVDKRVESKYGPPCPPCPAPEFLGGPSVFLFPPKPKDTLMISRTPEVTCVVVDVSQEDPEVQFNWYVDGVEVHNAKTKPREEQFNSTYRVVSVLTVLHQDWLNGKEYKCKVSNKGLPSSIEKTISKAKGQPREPQVYTLPPSQEEMTKNQVSLTCLVKGFYPSDIAVEWESNGQPENNYKTTPPVLDSDGSFFLYSRLTVDKSRWQEGNVFSCSVMHEALHNHYTQKSLSLSLGK

SEQ ID NO: 82 - protein, 445 aa, Artificial Sequence
  CHAIN: Heavy chain sequence of Hu33-6. IgG4P
KVQLVESGGGLVQPGGSLRLSCAASGFTFSSYAMSWVRQAPGKGLEWVATISGGGVDTYYQDNVQGRFTISRDNAKNSLYLQMNSLRAEDTAVYYCASPYGHGYFDVWGQGTTVTVSSASTKGPSVFPLAPCSRSTSESTAALGCLVKDYFPEPVTVSWNSGALTSGVHTFPAVLQSSGLYSLSSVVTVPSSSLGTKTYTCNVDHKPSNTKVDKRVESKYGPPCPPCPAPEFLGGPSVFLFPPKPKDTLMISRTPEVTCVVVDVSQEDPEVQFNWYVDGVEVHNAKTKPREEQFNSTYRVVSVLTVLHQDWLNGKEYKCKVSNKGLPSSIEKTISKAKGQPREPQVYTLPPSQEEMTKNQVSLTCLVKGFYPSDIAVEWESNGQPENNYKTTPPVLDSDGSFFLYSRLTVDKSRWQEGNVFSCSVMHEALHNHYTQKSLSLSLGK